European Patent Specification EP 4 457 366 B1, published February 4, 2026. Title: FLOW CELL SURFACE PATTERNING. Applicant: Illumina, Inc. The sequence listing filed with the application follows.

SEQUENCE LISTING (17 sequences)

SEQ ID NO: 1 - DNA, 28 bp, synthetic construct
  source 1..28: mol_type = other DNA
aatgatacggcgaccaccgagactacac

SEQ ID NO: 2 - DNA, 23 bp, synthetic construct
  source 1..23: mol_type = other DNA
caagcagaagacggcatacgaat

SEQ ID NO: 3 - DNA, 23 bp, synthetic construct
  source 1..23: mol_type = other DNA
caagcagaagacggcatacagat

SEQ ID NO: 4 - DNA, 35 bp, synthetic construct
  source 1..35: mol_type = other DNA
gctggcacgtccgaacgcttcgttaatccgttgag

SEQ ID NO: 5 - DNA, 35 bp, synthetic construct
  source 1..35: mol_type = other DNA
ctcaacggattaacgaagcgttcggacgtgccagc

SEQ ID NO: 6 - DNA, 35 bp, synthetic construct
  source 1..35: mol_type = other DNA
cgtcgtctgccatggcgcttcggtggatatgaact

SEQ ID NO: 7 - DNA, 35 bp, synthetic construct
  source 1..35: mol_type = other DNA
agttcatatccaccgaagcgccatggcagacgacg

SEQ ID NO: 8 - DNA, 35 bp, synthetic construct
  source 1..35: mol_type = other DNA
acggccgctaatatcaacgcgtcgaatccgcaact

SEQ ID NO: 9 - DNA, 35 bp, synthetic construct
  source 1..35: mol_type = other DNA
agttgcggattcgacgcgttgatattagcggccgt

SEQ ID NO: 10 - DNA, 34 bp, synthetic construct
  source 1..34: mol_type = other DNA
gccgcgttacgttagccggactattcgatgcagc

SEQ ID NO: 11 - DNA, 34 bp, synthetic construct
  source 1..34: mol_type = other DNA
gctgcatcgaatagtccggctaacgtaacgcggc

SEQ ID NO: 12 - DNA, 29 bp, synthetic construct
  source 1..29: mol_type = other DNA
  modified_base 23: mod_base = OTHER; note = uracil or allyl T
aatgatacggcgaccaccgaganctacac

SEQ ID NO: 13 - DNA, 24 bp, synthetic construct
  source 1..24: mol_type = other DNA
  modified_base 22: mod_base = OTHER; note = 8-oxoguanine
caagcagaagacggcatacganat

SEQ ID NO: 14 - DNA, 24 bp, synthetic construct
  source 1..24: mol_type = other DNA
  modified_base 20: mod_base = OTHER; note = 8-oxoguanine
caagcagaagacggcatacnagat

SEQ ID NO: 15 - DNA, 24 bp, synthetic construct
  source 1..24: mol_type = other DNA
  modified_base 20: mod_base = OTHER; note = 8-oxoguanine
  modified_base 22: mod_base = OTHER; note = 8-oxoguanine
caagcagaagacggcatacnanat

SEQ ID NO: 16 - DNA, 24 bp, synthetic construct
  source 1..24: mol_type = other DNA
aggaggaggaggaggaggaggagg

SEQ ID NO: 17 - DNA, 24 bp, synthetic construct
  source 1..24: mol_type = other DNA
cctcctcctcctcctcctcctcct